European Patent Specification EP 3 587 441 B9, published October 4, 2023. Title: Novel antibacterial protein EFAL-2 having lytic activity against Enterococcus faecium. Applicant: iNtRON Biotechnology, Co. Ltd. The sequence listing filed with the application follows.

SEQUENCE LISTING (2 sequences)

SEQ ID NO: 1 - DNA, 975 bp, Gene coding antibacterial protein EFAL-2
atgtacacaattgacactagtcagaagttagcacctaatgaaggctccagccaagtagctaaccctaactacattattttgcatgaaaccgctaacccaaacgctggtggactaaacaatgctaaatatatgaaacgtacatggtataacgcttacacagcttatatcgttggcgagggtaaagcttaccaagtaggtgaagatggttatgtacaatatggtgctggctcgtatgcaaacgctaacgcaccagtacaaattgagttagaccacaccacagacaaagcaatgtttcaaaagaactacaaagtatacgttgagttagcacgtgataaagctaaaaaatataacattcctttgacgcttgacacgccttataatcaacgtggtattaagtcacacttatgggtaactcaaaacatttggggtgaccactcagacccatatggttacttacaaagcatgggtatttctaaacagaaattagctcatgacttagctaacggttttggttctgatacaaacaatccagtaccaaacccaacaccatcaaacccacaaacagcacatgacaacgctgtcacaaaatctgcaccagttactaacggtaattacattggtaaacttgacgtgttcaaggaacaaccaaaaggacaattacgtattgctggttggaatgtggctgtaaatggtgctgacgcttaccgttatggttttgttttctacatggacgctaacactggtaaagaagtagctcgttcaatgagtaaaggaattgctagaccagatgtttcaaaagcctatggtttgccagttacaaacaaatatggacttgatacaactgtgcctatgagtaagttaaaaggtcacaaaatcattccaatgttcagacgaactaatgacccaagtggaaacactaaaggtggttcacatgatgtaatgttaccaaacatttatatcaatgtacctaaataa

SEQ ID NO: 2 - protein, 324 aa, antibacterial protein EFAL-2
MYTIDTSQKLAPNEGSSQVANPNYIILHETANPNAGGLNNAKYMKRTWYNAYTAYIVGEGKAYQVGEDGYVQYGAGSYANANAPVQIELDHTTDKAMFQKNYKVYVELARDKAKKYNIPLTLDTPYNQRGIKSHLWVTQNIWGDHSDPYGYLQSMGISKQKLAHDLANGFGSDTNNPVPNPTPSNPQTAHDNAVTKSAPVTNGNYIGKLDVFKEQPKGQLRIAGWNVAVNGADAYRYGFVFYMDANTGKEVARSMSKGIARPDVSKAYGLPVTNKYGLDTTVPMSKLKGHKIIPMFRRTNDPSGNTKGGSHDVMLPNIYINVPK